European Patent Specification EP 3 699 271 B1, published September 25, 2024. Title: PHYTIC ACID AS A STABILIZER FOR PHYTASE. Applicant: DANISCO US INC. GEBERT, Mark S. Application 2013-02-01. The sequence listing filed with the application follows.

SEQUENCE LISTING (12 sequences)

SEQ ID NO: 1 - protein, 413 aa, Artificial Sequence
  Synthetic construct: BP17, a variant phytase of Buttiauxella sp. comprising 12 amino acid substitutions compared to the wild type (SEQ ID NO:4), lacking the signal sequence (SEQ ID NO:12)
NDTPASGYQVEKVVILSRHGVRAPTKMTQTMRDVTPNTWPEWPVKLGYITPRGEHLISLMGGFYRQKFQQQGILSQGSCPTPNSIYVWTDVAQRTLKTGEAFLAGLAPQCGLTIHHQQNLEKADPLFHPVKAGICSMDKTQVQQAVEKEAQTPIDNLNQHYIPSLALMNTTLNFSKSPWCQKHSADKSCDLGLSMPSKLSIKDNGNEVSLDGAIGLSSTLAEIFLLEYAQGMPQAAWGNIHSEQEWALLLKLHNVYFDLMERTPYIARHKGTPLLQAISNALNPNATESKLPDISPDNKILFIAGHDTNIANIAGMLNMRWTLPGQPDNTPPGGALVFERLADKSGKQYVSVSMVYQTLEQLRSQTPLSLNQPAGSVQLKIPGCNDQTAEGYCPLSTFTRVVSQSVEPGCQLQ

SEQ ID NO: 2 - protein, 413 aa, Artificial Sequence; identical to SEQ ID NO: 1
  Synthetic construct: BP11, a variant phytase of Buttiauxella sp. comprising 11 amino acid substitutions compared to the wild type (SEQ ID NO: 4), lacking the signal sequence (SEQ ID NO: 12)

SEQ ID NO: 3 - protein, 413 aa, Artificial Sequence
  Synthetic construct: BP111, a variant phytase of Buttiauxella sp. comprising 21 amino acid substitutions compared to the wild type (SEQ ID NO:4), lacking the signal sequence (SEQ ID NO: 12)
NDTPASGYQVEKVVILSRHGVRAPTKMTQTMRDVTPNTWPEWPVKLGYITPRGEHLISLMGGFYRQKFQQQGILSQGSCPTPNSIYVWTDVDQRTLKTGEAFLAGLAPQCGLTIHHQQNLEKADPLFHPVKAGICSMDKTQVQQAVEKEAQTPIDNLNQHYIPSLALMNTTLNFSKSPWCQKHSADKSCDLGLSMPSKLSIKDNGNEVSLDGAIGLSSTLAEIFLLEYAQGMPQAAWGNIHSEQEWALLLKLHNVYFDLMERTPYIARHKGTPLLQAISNALNPNATESKLPDISPDNKILFIAGHDTNIANIAGMLNMRWTLPGQPDNTPPGGALVFERLADKSGKQYVSVSMVYQTLEQLRSQTPLSLNQPAGSVQLKIPGCNDQTAEGYCPLSTFTRVVSQSVEPGCQLQ

SEQ ID NO: 4 - protein, 413 aa, Buttiauxella sp.
  misc_feature: Wild type phytase encoded by Buttiauxella sp. strain P 1-29 deposited under accession number NCIMB 41248, lacking the signal sequence (SEQ ID NO: 12)
NDTPASGYQVEKVVILSRHGVRAPTKMTQTMRDVTPYTWPEWPVKLGYITPRGEHLISLMGGFYRQKFQQQGILPRGSCPTPNSIYVWTDVAQRTLKTGEAFLAGLAPQCGLTIHHQQNLEKADPLFHPVKAGICSMDKTQVQQAVEKEAQTPIDNLNQRYIPELALMNTILNFSKSPWCQKHSADKPCDLALSMPSKLSIKDNGNEVSLDGAIGLSSTLAEIFLLEYAQGMPQVAWGNIHSEQEWALLLKLHNVYFDLMERTPYIARHKGTPLLQAISNALNPNATESKLPDISPDNKILFIAGHDTNIANIAGMLNMRWTLPGQPDNTPPGGALVFERLADKSGKQYVSVSMVYQTLEQLRSQTPLSLNQPPGSVQLKIPGCNDQTAEGYCPLSTFTRVVSQSVEPGCQLQ

SEQ ID NO: 5 - protein, 413 aa, Artificial Sequence
  Synthetic construct: BP17 with an additional amino acid substitution E121T
NDTPASGYQVEKVVILSRHGVRAPTKMTQTMRDVTPNTWPEWPVKLGYITPRGEHLISLMGGFYRQKFQQQGILSQGSCPTPNSIYVWADVDQRTLKTGEAFLAGLAPQCGLTIHHQQNLEKADPLFHPVKAGTCSMDKTQVQQAVEKEAQTPIDNLNQHYIPFLALMNTTLNFSTSAWCQKHSADKSCDLGLSMPSKLSIKDNGNKVALDGAIGLSSTLAEIFLLEYAQGMPQAAWGNIHSEQEWASLLKLHNVQFDLMARTPYIARHNGTPLLQAISNALNPNATESKLPDISPDNKILFIAGHDTNIANIAGMLNMRWTLPGQPDNTPPGGALVFERLADKSGKQYVSVSMVYQTLEQLRSQTPLSLNQPAGSVQLKIPGCNDQTAEGYCPLSTFTRVVSQSVEPGCQLQ

SEQ ID NO: 6 - protein, 413 aa, Artificial Sequence
  Synthetic construct: BP17 with an additional amino acid substitution P394N
NDTPASGYQVEKVVILSRHGVRAPTKMTQTMRDVTPNTWPEWPVKLGYITPRGEHLISLMGGFYRQKFQQQGILSQGSCPTPNSIYVWTDVAQRTLKTGEAFLAGLAPQCGLTIHHQQNLEKADPLFHPVKAGICSMDKTQVQQAVEKEAQTPIDNLNQHYIPSLALMNTTLNFSKSPWCQKHSADKSCDLGLSMPSKLSIKDNGNEVSLDGAIGLSSTLAEIFLLEYAQGMPQAAWGNIHSEQEWALLLKLHNVYFDLMERTPYIARHKGTPLLQAISNALNPNATESKLPDISPDNKILFIAGHDTNIANIAGMLNMRWTLPGQPDNTPPGGALVFERLADKSGKQYVSVSMVYQTLEQLRSQTPLSLNQPAGSVQLKIPGCNDQTAEGYCNLSTFTRVVSQSVEPGCQLQ

SEQ ID NO: 7 - protein, 413 aa, Artificial Sequence
  Synthetic construct: BP17 with an additional amino acid substitution D386N
NDTPASGYQVEKVVILSRHGVRAPTKMTQTMRDVTPNTWPEWPVKLGYITPRGEHLISLMGGFYRQKFQQQGILSQGSCPTPNSIYVWTDVAQRTLKTGEAFLAGLAPQCGLTIHHQQNLEKADPLFHPVKAGICSMDKTQVQQAVEKEAQTPIDNLNQHYIPSLALMNTTLNFSKSPWCQKHSADKSCDLGLSMPSKLSIKDNGNEVSLDGAIGLSSTLAEIFLLEYAQGMPQAAWGNIHSEQEWALLLKLHNVYFDLMERTPYIARHKGTPLLQAISNALNPNATESKLPDISPDNKILFIAGHDTNIANIAGMLNMRWTLPGQPDNTPPGGALVFERLADKSGKQYVSVSMVYQTLEQLRSQTPLSLNQPAGSVQLKIPGCNNQTAEGYCPLSTFTRVVSQSVEPGCQLQ

SEQ ID NO: 8 - protein, 413 aa, Artificial Sequence
  Synthetic construct: BP17 with additional amino acid substitutions K202N and N204T
NDTPASGYQVEKVVILSRHGVRAPTKMTQTMRDVTPNTWPEWPVKLGYITPRGEHLISLMGGFYRQKFQQQGILSQGSCPTPNSIYVWTDVAQRTLKTGEAFLAGLAPQCGLTIHHQQNLEKADPLFHPVKAGICSMDKTQVQQAVEKEAQTPIDNLNQHYIPSLALMNTTLNFSKSPWCQKHSADKSCDLGLSMPSKLSINDTGNEVSLDGAIGLSSTLAEIFLLEYAQGMPQAAWGNIHSEQEWALLLKLHNVYFDLMERTPYIARHKGTPLLQAISNALNPNATESKLPDISPDNKILFIAGHDTNIANIAGMLNMRWTLPGQPDNTPPGGALVFERLADKSGKQYVSVSMVYQTLEQLRSQTPLSLNQPAGSVQLKIPGCNDQTAEGYCPLSTFTRVVSQSVEPGCQLQ

SEQ ID NO: 9 - protein, 413 aa, Artificial Sequence
  Synthetic construct: BP17 with additional amino acid substitutions Q151N and P153S
NDTPASGYQVEKVVILSRHGVRAPTKMTQTMRDVTPNTWPEWPVKLGYITPRGEHLISLMGGFYRQKFQQQGILSQGSCPTPNSIYVWTDVAQRTLKTGEAFLAGLAPQCGLTIHHQQNLEKADPLFHPVKAGICSMDKTQVQQAVEKEANTSIDNLNQHYIPSLALMNTTLNFSKSPWCQKHSADKSCDLGLSMPSKLSIKDNGNEVSLDGAIGLSSTLAEIFLLEYAQGMPQAAWGNIHSEQEWALLLKLHNVYFDLMERTPYIARHKGTPLLQAISNALNPNATESKLPDISPDNKILFIAGHDTNIANIAGMLNMRWTLPGQPDNTPPGGALVFERLADKSGKQYVSVSMVYQTLEQLRSQTPLSLNQPAGSVQLKIPGCNDQTAEGYCPLSTFTRVVSQSVEPGCQLQ

SEQ ID NO: 10 - protein, 413 aa, Artificial Sequence
  Synthetic construct: BP17 with an additional amino acid substitution P373T
NDTPASGYQVEKVVILSRHGVRAPTKMTQTMRDVTPNTWPEWPVKLGYITPRGEHLISLMGGFYRQKFQQQGILSQGSCPTPNSIYVWTDVAQRTLKTGEAFLAGLAPQCGLTIHHQQNLEKADPLFHPVKAGICSMDKTQVQQAVEKEAQTPIDNLNQHYIPSLALMNTTLNFSKSPWCQKHSADKSCDLGLSMPSKLSIKDNGNEVSLDGAIGLSSTLAEIFLLEYAQGMPQAAWGNIHSEQEWALLLKLHNVYFDLMERTPYIARHKGTPLLQAISNALNPNATESKLPDISPDNKILFIAGHDTNIANIAGMLNMRWTLPGQPDNTPPGGALVFERLADKSGKQYVSVSMVYQTLEQLRSQTPLSLNQTAGSVQLKIPGCNDQTAEGYCPLSTFTRVVSQSVEPGCQLQ

SEQ ID NO: 11 - protein, 413 aa, Artificial Sequence
  Synthetic construct: BP17 with an additional amino acid substitution Q76N
NDTPASGYQVEKVVILSRHGVRAPTKMTQTMRDVTPNTWPEWPVKLGYITPRGEHLISLMGGFYRQKFQQQGILSNGSCPTPNSIYVWTDVAQRTLKTGEAFLAGLAPQCGLTIHHQQNLEKADPLFHPVKAGICSMDKTQVQQAVEKEAQTPIDNLNQHYIPSLALMNTTLNFSKSPWCQKHSADKSCDLGLSMPSKLSIKDNGNEVSLDGAIGLSSTLAEIFLLEYAQGMPQAAWGNIHSEQEWALLLKLHNVYFDLMERTPYIARHKGTPLLQAISNALNPNATESKLPDISPDNKILFIAGHDTNIANIAGMLNMRWTLPGQPDNTPPGGALVFERLADKSGKQYVSVSMVYQTLEQLRSQTPLSLNQPAGSVQLKIPGCNDQTAEGYCPLSTFTRVVSQSVEPGCQLQ

SEQ ID NO: 12 - protein, 33 aa, Buttiauxella sp.
  misc_feature: Signal sequence for wild type (SEQ ID NO: 4)
MTISAFNRKKLTLHPGLFVALSAIFSLGSTAYA